European Patent Application EP 4 421 165 A9, published May 21, 2025. Title: OILSEED RAPE GREEN REVOLUTION GENE BGR AND USE THEREOF. Applicant: 中国科学院遗传与发育生物学研究所. Application CN 2022111773991, filed September 26, 2022. The sequence listing filed with the application follows.

SEQUENCE LISTING (36 sequences)

SEQ ID NO: 1 - DNA, 2870 bp, Brassica. rapa
  source 1..2870: mol_type = genomic DNA
atgacctcactatcattggggcctcagcctccggctactgctcagccgccgcagcttcgcgacggagatgcttccaggcgtcgttccgatatggatacagacaaggttgctccctccctctccctctctctctctatccactttaacgtttggtgaacaaattgcatttcgattggctattgtagatctcgcttagatctagcttcgatttcactttgttttgcggtttctcagcgaatcgatctgtgttttctcttgctatcgtttcgcgttccttgatttgagctcactcgtcggagttcgtagtagctatagctagtcttactattcagctgaatgtttcaaccaatcatagtgaagatcttcagctagattttgattactagtattagggtgaaattcgatttcacaggagtatggagacgatttagatcttaattactagattgtttaactaatcacacgcttgttccatgactgtaagtgatttggtgtatttgatttacatttgtttgttatttacttgattggactctgaactaggcctttgactgttcttggatttgaagatttcatatgtttaaaaaatgattttgtctactgattgttgtcatatcgtaatctcatgtttattgtttacagaagaatagtttaatgatatggtgaggttttggttgcaggatatgtctgctgctgtgatagagggaaacgatgctgttacaggccacatcatttctactacaattggaggcaaaaacggtgaacctaaacaggtttgagttcctttctttgtttgaaatcttcaattgtccttattagtagtcattgctaatgattatatagcttttccacttatagcttaaaacaataactaaacagagactctttgtggttcatttattaccaactttaagtaggctacagctactcacttatgttttactcattctgtttttttacagaccattagttacatggcggaacgggttgttggacaaggatcattcggaatcgtgttccaggtacctttgtgcttttcactcgctgttatcatttgtaggcaatagctttcttctttcttttctgatcggattattaccttaccattgtaggccaagtgcttggaaactggagaatctgtagccattaagaaggtcttgcaagaccggcgctacaagaatcgtgagctgcagttgatgcgactaatggaccacccaaatgtggtttccttgaagcattgtttcttctctactacgagtagagatgagctcttcctcaatctcgttatggagtatgtacccgagactttgtaccgggttctgaagcactatactagttcaagccagagaatgcctattttctatgtcaaactctacacataccaagtatgcattgttatttatctgtttccctttcaggcagtatctctctttgttgattctaaaacgggtaagaatacttttttttctgcagatcttcagaggcttggcttatatccatactgttcctggtgtctgtcacagagatgtgaaaccacaaaatcttttggtatgttaattctgttttgggtttgtcttcggcgatctttactagattgtaatctaataatttggtatgttctgtaggttgatccccttactcatcagtgtaagctgtgtgattttggaagtgcaaaagtattggtaaggagctttacctttaatatcctgctttgcttatttcaactgtgtatgtgttctgtctcatgaaatcattgcaacacatgattattcggattaggtgaaaggtgaagcaaacatatcatacatctgctctcggtattaccgagctccagagctgatctttggggccacagagtatacatcctccatagacatatggtctgctggttgtgttttggcagagctccttcttggccaggttagtgtaaactattttatctgtttaaatataactctagaatgttccgctatcatttttgatatatatataatttttttatctgtcagccgttgttcccgggagaaaattctgtggaccagctggtggagatcatcaaggtgaagtttcattttgatcagatgttaccttactgtcgtattctgttttgtatataaaactcatataatcttatagatttgtaatgatatatgtgctgcgtttgtttaggttcttggtactccaacccgaaaagaaatccgatgcatgaatccaaactacacagacttcagattcccgcaaatcaaagcacacccgtggcataaggtatctaatatgcttgtcactttctaacatgtcggataatacaatggcttaatagttggctcgctacctaattcctctatgacatccaggttttccataagaggatgcctcctgaagccattgacctcgcatctcggcttcttcagtattcaccgagcctgcgttacactgcggtcagtatatttaagccacttagtactcttacttgttagagtgattctctctggattcttcagtgatgctgatgttttctttttaactgacatttgtttgttttatgtgtgtaaaagcttgaagcatgtgcacatccgtttttcaatgaactccgtgagcccaatgctcgtcttccaaacggccgacctctaccagccttgttcaacttcaaacaagaggtacgtcaatcacagcaaaaaaaaggaagtaatatagctccaaaccataactagaatgttcagttttaaacagttacctaatctgtaatctctctctctctattcgaatgttcataacagttagctggggcttcaccagagctgataaacaggctcataccggagcacataaggcgacagatgagtggaggcttcccatcacagcctggtcat

SEQ ID NO: 2 - DNA, 2870 bp, Brassica. rapa
  source 1..2870: mol_type = genomic DNA
atgacctcactatcattggggcctcagcctccggctactgctcagccgccgcagcttcgcgacggagatgcttccaggcgtcgttccgatatggatacagacaaggttgctccctccctctccctctctctctctatccactttaacgtttggtgaacaaattgcatttcgattggctattgtagatctcgcttagatctagcttcgatttcactttgttttgcggtttctcagcgaatcgatctgtgttttctcttgctatcgtttcgcgttccttgatttgagctcactcgtcggagttcgtagtagctatagctagtcttactattcagctgaatgtttcaaccaatcatagtgaagatcttcagctagattttgattactagtattagggtgaaattcgatttcacaggagtatggagacgatttagatcttaattactagattgtttaactaatcacacgcttgttccatgactgtaagtgatttggtgtatttgatttacatttgtttgttatttacttgattggactctgaactaggcctttgactgttcttggatttgaagatttcatatgtttaaaaaatgattttgtctactgattgttgtcatatcgtaatctcatgtttattgtttacagaagaatagtttaatgatatggtgaggttttggttgcaggatatgtctgctgctgtgatagagggaaacgatgctgttacaggccacatcatttctactacaattggaggcaaaaacggtgaacctaaacaggtttgagttcctttctttgtttgaaatcttcaattgtccttattagtagtcattgctaatgattatatagcttttccacttatagcttaaaacaataactaaacagagactctttgtggttcatttattaccaactttaagtaggctacagctactcacttatgttttactcattctgtttttttacagaccattagttacatggcggaacgggttgttggacaaggatcattcggaatcgtgttccaggtacctttgtgcttttcactcgctgttatcatttgtaggcaatagctttcttctttcttttctgatcggattattaccttaccattgtaggccaagtgcttggaaactggagaatctgtagccattaagaaggtcttgcaagaccggcgctacaagaatcgtgagctgcagttgatgcgactaatggaccacccaaatgtggtttccttgaagcattgtttcttctctactacgagtagagatgagctcttcctcaatctcgttatggagtatgtacccgagactttgtaccgggttctgaagcactatactagttcaagccagagaatgcctattttctatgtcaaactctacacataccaagtatgcattgttatttatctgtttccctttcaggcagtatctctctttgttgattctaaaacgggtaagaatacttttttttctgcagatcttcagaggcttggcttatatccatactgttcctggtgtctgtcacagagatgtgaaaccacaaaatcttttggtatgttaattctgttttgggtttgtcttcggcgatctttactagattgtaatctaataatttggtatgttctgtaggttgatccccttactcatcagtgtaagctgtgtgattttggaagtgcaaaagtattggtaaggagctttacctttaatatcctgctttgcttatttcaactgtgtatgtgttctgtctcatgaaatcattgcaacacatgattattcggattaggtgaaaggtgaagcaaacatatcatacatctgctctcggtattaccgagctccagagctgatctttggggccacagagtatacatcctccatagacatatggtctgctggttgtgttttggcagagctccttcttggccaggttagtgtaaactattttatctgtttaaatataactctagaatgttccgctatcatttttgatatatatataatttttttatctgtcagccgttgttcccgggagaaaattctgtggaccagctggtggagatcatcaaggtgaagtttcattttgatcagatgttaccttactgtcgtattctgttttgtatataaaactcatataatcttatagatttgtaatgatatatgtgctgcgtttgtttaggttcttggtactccaacccgagaagaaatccgatgcatgaatccaaactacacagacttcagattcccgcaaatcaaagcacacccgtggcataaggtatctaatatgcttgtcactttctaacatgtcggataatacaatggcttaatagttggctcgctacctaattcctctatgacatccaggttttccataagaggatgcctcctgaagccattgacctcgcatctcggcttcttcagtattcaccgagcctgcgttacactgcggtcagtatatttaagccacttagtactcttacttgttagagtgattctctctggattcttcagtgatgctgatgttttctttttaactgacatttgtttgttttatgtgtgtaaaagcttgaagcatgtgcacatccgtttttcaatgaactccgtgagcccaatgctcgtcttccaaacggccgacctctaccagccttgttcaacttcaaacaagaggtacgtcaatcacagcaaaaaaaaggaagtaatatagctccaaaccataactagaatgttcagttttaaacagttacctaatctgtaatctctctctctctattcgaatgttcataacagttagctggggcttcaccagagctgataaacaggctcataccggagcacataaggcgacagatgagtggaggcttcccatcacagcctggtcat

SEQ ID NO: 3 - DNA, 1230 bp, Brassica. rapa
  source 1..1230: mol_type = other DNA
atgacctcactatcattggggcctcagcctccggctactgctcagccgccgcagcttcgcgacggagatgcttccaggcgtcgttccgatatggatacagacaaggatatgtctgctgctgtgatagagggaaacgatgctgttacaggccacatcatttctactacaattggaggcaaaaacggtgaacctaaacagaccattagttacatggcggaacgggttgttggacaaggatcattcggaatcgtgttccaggccaagtgcttggaaactggagaatctgtagccattaagaaggtcttgcaagaccggcgctacaagaatcgtgagctgcagttgatgcgactaatggaccacccaaatgtggtttccttgaagcattgtttcttctctactacgagtagagatgagctcttcctcaatctcgttatggagtatgtacccgagactttgtaccgggttctgaagcactatactagttcaagccagagaatgcctattttctatgtcaaactctacacataccaaatcttcagaggcttggcttatatccatactgttcctggtgtctgtcacagagatgtgaaaccacaaaatcttttggttgatccccttactcatcagtgtaagctgtgtgattttggaagtgcaaaagtattggtgaaaggtgaagcaaacatatcatacatctgctctcggtattaccgagctccagagctgatctttggggccacagagtatacatcctccatagacatatggtctgctggttgtgttttggcagagctccttcttggccagccgttgttcccgggagaaaattctgtggaccagctggtggagatcatcaaggttcttggtactccaacccgaaaagaaatccgatgcatgaatccaaactacacagacttcagattcccgcaaatcaaagcacacccgtggcataaggttttccataagaggatgcctcctgaagccattgacctcgcatctcggcttcttcagtattcaccgagcctgcgttacactgcgcttgaagcatgtgcacatccgtttttcaatgaactccgtgagcccaatgctcgtcttccaaacggccgacctctaccagccttgttcaacttcaaacaagagttagctggggcttcaccagagctgataaacaggctcataccggagcacataaggcgacagatgagtggaggcttcccatcacagcctggtcat

SEQ ID NO: 4 - protein, 410 aa, Brassica. rapa
MTSLSLGPQPPATAQPPQLRDGDASRRRSDMDTDKDMSAAVIEGNDAVTGHIISTTIGGKNGEPKQTISYMAERVVGQGSFGIVFQAKCLETGESVAIKKVLQDRRYKNRELQLMRLMDHPNVVSLKHCFFSTTSRDELFLNLVMEYVPETLYRVLKHYTSSSQRMPIFYVKLYTYQIFRGLAYIHTVPGVCHRDVKPQNLLVDPLTHQCKLCDFGSAKVLVKGEANISYICSRYYRAPELIFGATEYTSSIDIWSAGCVLAELLLGQPLFPGENSVDQLVEIIKVLGTPTRKEIRCMNPNYTDFRFPQIKAHPWHKVFHKRMPPEAIDLASRLLQYSPSLRYTALEACAHPFFNELREPNARLPNGRPLPALFNFKQELAGASPELINRLIPEHIRRQMSGGFPSQPGH

SEQ ID NO: 5 - DNA, 1230 bp, Brassica. rapa
  source 1..1230: mol_type = other DNA
atgacctcactatcattggggcctcagcctccggctactgctcagccgccgcagcttcgcgacggagatgcttccaggcgtcgttccgatatggatacagacaaggatatgtctgctgctgtgatagagggaaacgatgctgttacaggccacatcatttctactacaattggaggcaaaaacggtgaacctaaacagaccattagttacatggcggaacgggttgttggacaaggatcattcggaatcgtgttccaggccaagtgcttggaaactggagaatctgtagccattaagaaggtcttgcaagaccggcgctacaagaatcgtgagctgcagttgatgcgactaatggaccacccaaatgtggtttccttgaagcattgtttcttctctactacgagtagagatgagctcttcctcaatctcgttatggagtatgtacccgagactttgtaccgggttctgaagcactatactagttcaagccagagaatgcctattttctatgtcaaactctacacataccaaatcttcagaggcttggcttatatccatactgttcctggtgtctgtcacagagatgtgaaaccacaaaatcttttggttgatccccttactcatcagtgtaagctgtgtgattttggaagtgcaaaagtattggtgaaaggtgaagcaaacatatcatacatctgctctcggtattaccgagctccagagctgatctttggggccacagagtatacatcctccatagacatatggtctgctggttgtgttttggcagagctccttcttggccagccgttgttcccgggagaaaattctgtggaccagctggtggagatcatcaaggttcttggtactccaacccgagaagaaatccgatgcatgaatccaaactacacagacttcagattcccgcaaatcaaagcacacccgtggcataaggttttccataagaggatgcctcctgaagccattgacctcgcatctcggcttcttcagtattcaccgagcctgcgttacactgcgcttgaagcatgtgcacatccgtttttcaatgaactccgtgagcccaatgctcgtcttccaaacggccgacctctaccagccttgttcaacttcaaacaagagttagctggggcttcaccagagctgataaacaggctcataccggagcacataaggcgacagatgagtggaggcttcccatcacagcctggtcat

SEQ ID NO: 6 - protein, 410 aa, Brassica. rapa
MTSLSLGPQPPATAQPPQLRDGDASRRRSDMDTDKDMSAAVIEGNDAVTGHIISTTIGGKNGEPKQTISYMAERVVGQGSFGIVFQAKCLETGESVAIKKVLQDRRYKNRELQLMRLMDHPNVVSLKHCFFSTTSRDELFLNLVMEYVPETLYRVLKHYTSSSQRMPIFYVKLYTYQIFRGLAYIHTVPGVCHRDVKPQNLLVDPLTHQCKLCDFGSAKVLVKGEANISYICSRYYRAPELIFGATEYTSSIDIWSAGCVLAELLLGQPLFPGENSVDQLVEIIKVLGTPTREEIRCMNPNYTDFRFPQIKAHPWHKVFHKRMPPEAIDLASRLLQYSPSLRYTALEACAHPFFNELREPNARLPNGRPLPALFNFKQELAGASPELINRLIPEHIRRQMSGGFPSQPGH

SEQ ID NO: 7 - DNA, 1234 bp, Brassica. rapa
  source 1..1234: mol_type = other DNA
atgttcgaaatctacaaataaggagccataaaacaaaatattccaagaaatggactgcgatcgtccatgtgctacatccatggcccctatcttaagacttttaaacgtctctcgtattgaaccaaatgttaaaacccgttgaaaaggtacccatcttgctcatataaacgaagtttttcttagataacatcgaaaaaaattgtagattaaagatttcaaaccggacacgaaatctagtttgagtctgtatgtattaaagtaaaaagtaacaagttgaaaataagattatggtaatctgtaaatgttcacttgggaacaaatgcagtaaaaaaacgaatttactaaaagaggttccacagaaaaggctaaggcaaagcctattaccattcatgccatgtctaaattatttcgaataagtgtccaagcactttttttccctctaatgcttcttccgtcaaaagatgatcttttgcgatatactactaattggtcaatcttcaacaaaacatggtattattatataaaattgattttatttttatatatgacaaataatttgacatttctaggtcagaaagcgggaaatacaaacaatttgatgatgctcttttctaaatccagtaaaaaaaaactaattttacaaatctaaaaatatgcaaatggtatcagttgttacccagtcaaaatatgaaaacaatttatgtccatcgtttaaagaaaaatatattaaatatccggagtttctttttgtagccaccattatattgcaactaattgcaaggttatcagactttccagctcacaattaaactgatgagaggtgcgtaaactaatagactagccttctaataggagcgtttctattacgcgctctgttcacgcgtgggtcatccttttcaaacatactatactagttgttacttgttacccaaaatgtaaatacatgccatgtccttactaggcagtatatagaaattagttcgttttaatgaatctgtaacaatactaacttctataattaattgcaaggttatccacccttgagagcttatgaaactgacgaggaagatattcgcgttctcattggtgcgtttcgtgtacgcgctttcttgacgcgtggaggatatacgaagttcttttaataatacaaagagagagagaggggaaagatagtctttactcttcagtggtgggtagagagcgaaagttagagagagagagagaagaatagcac

SEQ ID NO: 8 - DNA, 1140 bp, Brassica napus
  source 1..1140: mol_type = genomic DNA
atggctgacgatagggagatgccggctgctgtagttgatggacatgaccaagtcactggccacataatctccaccaccatcggtggtaaaaacggagaacctaaacagacaataagttacatggcggagcgagttgtcggaacaggctccttcgggatagtgttccaggcgaagtgtctggagactggagaaaccgtggcgataaagaaggtgttgcaagacaggaggtacaagaaccgggagcttcagctgatgcgtgtgatggaccatcctaatgttgtttgtctgaagcattgcttcttctcgaccacgagtaaagacgagctgtttcttaacttggttatggagtatgtccctgagagtttgtaccgagttctgaaacattacagcactgctaaccagaggatgccgcttgtctacgttaaactctatatgtaccagatcttcagaggacttgcttacattcacaatgttgctggagtttgtcacagagatctaaagcctcagaatcttctggttgatcctcttactcatcaagtcaagatctgtgattttggcagtgctaaacagcttgttaaaggtgaagccaacatctcttacatatgctcacggttctaccgtgcacctgaactcatatttggtgccactgagtacacaacttccattgatatctggtctgctggttgtgttctcgctgagcttcttcttggtcagccactattccctggagaaaatgctgtggatcagctcgttgaaataatcaaagttcttggtacaccaactcgagaagagatccgttgtatgaatccacactacacagacttcaggttcccgcagataaaggcacatccttggcacaagattttccacaaaaggatgcctccagaagcaattgattttgcttcaaggctgcttcagtactctccaagtcttagatgcacagcgcttgaagcttgtgcacatccgttctttgatgagctgagagaaccaaatgctcgtttaccaaacggacggcctttcccacctctcttcaacttcaaacaagaggtagctggagcttcacctgagctggtcaacaagttgattccagaccatatcaagaggcagttgggtctaagcttcttgaatcagtctggaact

SEQ ID NO: 9 - protein, 380 aa, Brassica napus
MADDREMPAAVVDGHDQVTGHIISTTIGGKNGEPKQTISYMAERVVGTGSFGIVFQAKCLETGETVAIKKVLQDRRYKNRELQLMRVMDHPNVVCLKHCFFSTTSKDELFLNLVMEYVPESLYRVLKHYSTANQRMPLVYVKLYMYQIFRGLAYIHNVAGVCHRDLKPQNLLVDPLTHQVKICDFGSAKQLVKGEANISYICSRFYRAPELIFGATEYTTSIDIWSAGCVLAELLLGQPLFPGENAVDQLVEIIKVLGTPTREEIRCMNPHYTDFRFPQIKAHPWHKIFHKRMPPEAIDFASRLLQYSPSLRCTALEACAHPFFDELREPNARLPNGRPFPPLFNFKQEVAGASPELVNKLIPDHIKRQLGLSFLNQSGT

SEQ ID NO: 10 - DNA, 1140 bp, Brassica napus
  source 1..1140: mol_type = genomic DNA
atggctgacgataaggagatgccggctgctgtagttgatggacatgaccaagtcactggtcacataatctccaccacaataggaggtaaaaacggagaacctaaacagactataagttacatggcggagcgagtcgtcggcacaggctccttcgggatagtgttccaagcaaagtgtttggagacaggagaaaccgtggcgataaagaaggttttgcaagacaggagatacaagaaccgagagcttcagctgatgcgtgtgatggaccatccgaacgtggttcgtttgaaacattgcttcttctcgaccacgagtaaagacgagcttttccttaatctggttatggagtatgtccctgagagcttgtaccgtgttctgaaacattacagcactgcgaaccagagaatgcctcttgtctacgttaaactctacatgtaccagatctttaggggacttgcttacgttcacaatgttgctggagtttgccatagagatctaaagccgcagaatcttctggttgatcctcttacacatcaagtcaagatatgtgactttggtagtgcgaaacagcttgttaaaggtgaagccaacatatcttacatatgttcaagattctaccgtgcacctgaacttatattcggtgctaccgagtacacaacttcaattgatatctggtctgctggttgtgtccttgctgagcttcttcttggtcagccattattccctggagagaatgctgttgatcagctagttgaaatcatcaaagttcttggtacaccaactcgagaagagatccgttgtatgaatccacactacacagactttaggttcccacagattaaagcacatccttggcacaagattttccataaacggatgcctccagaagctattgattttgcgtcaaggctgcttcagtactctcctagtcttagatgcacagcgctggaagcttgtgcacatccgttctttgatgaactgagagaaccaaatgctcgtttaccaaacggacggcctttcccgcctctcttcaacttcaaacaggaggtagctggagcatcacctgagctggtcaacaagttgattccagaccatatcaagagacagttgggtctaagtttcttgaatcagtctggaact

SEQ ID NO: 11 - protein, 380 aa, Brassica napus
MADDKEMPAAVVDGHDQVTGHIISTTIGGKNGEPKQTISYMAERVVGTGSFGIVFQAKCLETGETVAIKKVLQDRRYKNRELQLMRVMDHPNVVRLKHCFFSTTSKDELFLNLVMEYVPESLYRVLKHYSTANQRMPLVYVKLYMYQIFRGLAYVHNVAGVCHRDLKPQNLLVDPLTHQVKICDFGSAKQLVKGEANISYICSRFYRAPELIFGATEYTTSIDIWSAGCVLAELLLGQPLFPGENAVDQLVEIIKVLGTPTREEIRCMNPHYTDFRFPQIKAHPWHKIFHKRMPPEAIDFASRLLQYSPSLRCTALEACAHPFFDELREPNARLPNGRPFPPLFNFKQEVAGASPELVNKLIPDHIKRQLGLSFLNQSGT

SEQ ID NO: 12 - DNA, 1140 bp, Brassica napus
  source 1..1140: mol_type = genomic DNA
atggctgacgataaggaggtgccgggtgctgtagttaacggacacgatcacgtcactggccacataatctccacaactatcggaggcaaaaacggagaaccaaaacagacgataagttacatggcggagcgtgtcgtcggaacaggctcattcgggatagtcttccaggcgaagtgtttggagaccggagaaaccgtggcgataaagaaggttctgcaagacaggaggtacaagaaccgagagcttcagctgatgcgtgttatggaccatcctaatgtggtttgtttgaagcattgcttcttctccaccactagtaaagacgagctgtttctcaacttggttatggagtatgtacccgagagcttgtaccgtgttctgaaacattacagcactgctaaccagagaatgcctcttgtctatgttaaactctacatgtaccagatcttcaggggacttgcttatatgcacaatgttgctgaagtttgtcacagagatctaaagcctcaaaatcttctggttgatcctcttactcatcaagtcaagatctgtgactttggcagtgctaaacagcttgttaaaggtgaagccaacatctcttacatatgttcaagattctaccgtgcaccagagctcatatttggtgccactgagtacacaacttccattgatatctggtctgctggttgtgttcttgctgagcttctccttggtcagccattattccctggagaaaatgctgtggatcagctcgttgaaatcatcaaagttcttggtacaccaactcgagaagagatccgttgcatgaatccacattacacggactttaggttcccacagataaaggcacacccttggcacaagattttccataaaaggatgcctccagaagcgattgatttcgcatcgaggctgcttcagtactctccaagtcttagatgcacagctcttgaagcttgtgcacatccgttctttgatgaactgagagaaccaaatgctcgtttaccaaacggacggcctttcccgccaatcttcaacttcaaacaagaggtagctggagcatcacctgagctggtcaacaagttgattccggaccatatcaagagacagttgggtctaagtttcttgaatcagtctggaact

SEQ ID NO: 13 - protein, 380 aa, Brassica napus
MADDKEVPGAVVNGHDHVTGHIISTTIGGKNGEPKQTISYMAERVVGTGSFGIVFQAKCLETGETVAIKKVLQDRRYKNRELQLMRVMDHPNVVCLKHCFFSTTSKDELFLNLVMEYVPESLYRVLKHYSTANQRMPLVYVKLYMYQIFRGLAYMHNVAEVCHRDLKPQNLLVDPLTHQVKICDFGSAKQLVKGEANISYICSRFYRAPELIFGATEYTTSIDIWSAGCVLAELLLGQPLFPGENAVDQLVEIIKVLGTPTREEIRCMNPHYTDFRFPQIKAHPWHKIFHKRMPPEAIDFASRLLQYSPSLRCTALEACAHPFFDELREPNARLPNGRPFPPIFNFKQEVAGASPELVNKLIPDHIKRQLGLSFLNQSGT

SEQ ID NO: 14 - DNA, 1140 bp, Brassica napus
  source 1..1140: mol_type = genomic DNA
atggctgacgataaggaggtgcctgctgctgtagttaacggacacgatcaagtcactggccacataatctccacaactatcggaggcaaaaacggagaaccaaaacagacgataagttacatggcggagcgagtcgtcggaacaggctccttcgggatagtcttccaggccaagtgtttggagaccggagaaaccgtggcgataaagaaggttctgcaagacaggaggtacaagaaccgagagcttcagctgatgcgcgtcatggaccatcctaatgtggtttgtttgaagcattgcttcttctccaccactagtaaagacgagctgtttctcaacttggttatggagtatgtacccgagagcttgtaccgtgttctgaaacattacagcactgccaaccagagaatgcctcttgtctatgttaaactctacatgtaccagatcttcaggggacttgcttatatgcacaatgttgctggagtttgtcacagagatctaaagcctcaaaatcttctggttgatcctctgactcatcaagtcaagatctgtgactttgggagtgctaaacagcttgttaaaggtgaagccaacatctcttacatatgttcaagattctaccgtgcacccgagctcatattcggtgccaccgagtacacaacttccattgatatctggtctgctggttgtgttcttgctgagcttcttctcggtcagccattattccctggagaaaatgctgtggatcagcttgttgaaatcatcaaagttcttggtacaccaactcgagaagagatccgttgtatgaatccacattacacagactttaggttccctcagataaaggcacacccttggcacaagattttccataaaaggatgcctccagaagctattgatttcgcatcaaggctgcttcagtactctccaagtcttagatgcacagcgctggaagcatgtgcacatccgttctttgatgagctcagagaaccaaatgctcgtttaccaaacggacggcctttcccgcctatcttcaacttcaaacaagaggtagctggagcatcacctgagctggtcaacaagttgattccagaccatatcaagagacagttgggtctgagtttcttgaatcagtctggaact

SEQ ID NO: 15 - protein, 380 aa, Brassica napus
MADDKEVPAAVVNGHDQVTGHIISTTIGGKNGEPKQTISYMAERVVGTGSFGIVFQAKCLETGETVAIKKVLQDRRYKNRELQLMRVMDHPNVVCLKHCFFSTTSKDELFLNLVMEYVPESLYRVLKHYSTANQRMPLVYVKLYMYQIFRGLAYMHNVAGVCHRDLKPQNLLVDPLTHQVKICDFGSAKQLVKGEANISYICSRFYRAPELIFGATEYTTSIDIWSAGCVLAELLLGQPLFPGENAVDQLVEIIKVLGTPTREEIRCMNPHYTDFRFPQIKAHPWHKIFHKRMPPEAIDFASRLLQYSPSLRCTALEACAHPFFDELREPNARLPNGRPFPPIFNFKQEVAGASPELVNKLIPDHIKRQLGLSFLNQSGT

SEQ ID NO: 16 - DNA, 1140 bp, Brassica napus
  source 1..1140: mol_type = genomic DNA
atggctgccgataaggagatgccagctgctgtagttgctgggcatgatcaagtcactggtcacataatctccaccacaataggaggaaaaaacggagaacctaaacagacaataagttacatggcggagcgagtcgtcggcacaggttccttcgggatagtgttccaagcaaagtgtttggagacaggagaaaccgtagcgataaagaaagttctgcaagacaggagatacaagaaccgagagcttcagctgatgcgcgtgatggaccatccgaacgtggttcgtttgaagcattgcttcttctcgaccacgagtaaagacgagcttttccttaacttggttatggagtatgtccccgagagcttgtaccgtgttctcaaacattacagcaccgcgaaccagagaatgcctcttgtctacgttaaactctacatgtaccagatctttaggggacttgcttacgttcacaatgttgctggtgtttgccatagagatctaaagcctcaaaatcttctggttgatcctctaactcatcaagtcaagatctgtgactttggcagtgcgaaacagcttgttaaaggtgaagccaacatttcttacatatgttcaagattctaccgagcacctgaactcatatttggtgccactgagtacacaacatcaattgatatctggtctgctggttgtgtcctcgctgagcttcttcttggtcagccattattccctggagagaatgctgttgatcagctagttgaaatcatcaaagttcttggtacaccaactcgagaagagatccgttgtatgaatccacactacacagactttaggttcccgcagataaaagcacatccttggcacaagattttccacaaaagaatgcctccagaagctcttgattttgcgtcaaggctgcttcagtactctcctagtcttagatgcacagcgctggaagcttgtgcacatcctttctttgatgaactgagagaaccaaatgcttgtttaccaaacggacggcctttcccgcctctcttcaacttcaaacaggaggttgctggagcatcacctgagctggtgaacaagttgattccagaccatatcaagagacaattgggtctaagtttcttgaatcagtctggaact

SEQ ID NO: 17 - protein, 380 aa, Brassica napus
MAADKEMPAAVVAGHDQVTGHIISTTIGGKNGEPKQTISYMAERVVGTGSFGIVFQAKCLETGETVAIKKVLQDRRYKNRELQLMRVMDHPNVVRLKHCFFSTTSKDELFLNLVMEYVPESLYRVLKHYSTANQRMPLVYVKLYMYQIFRGLAYVHNVAGVCHRDLKPQNLLVDPLTHQVKICDFGSAKQLVKGEANISYICSRFYRAPELIFGATEYTTSIDIWSAGCVLAELLLGQPLFPGENAVDQLVEIIKVLGTPTREEIRCMNPHYTDFRFPQIKAHPWHKIFHKRMPPEALDFASRLLQYSPSLRCTALEACAHPFFDELREPNACLPNGRPFPPLFNFKQEVAGASPELVNKLIPDHIKRQLGLSFLNQSGT

SEQ ID NO: 18 - DNA, 1233 bp, Brassica napus
  source 1..1233: mol_type = genomic DNA
atgacatcctccataccattgggtcatcagcctccgtgtctagctccgcagccgccgccgcagctgcgcgacggagatgctttgaaacgtcgtcctgatatggatacagacaaggatatgtctgctgctgttatagagggcaatgatgctgttaccggtcacatcatttctactaccatcggaggcaaaaacggcgaacctaaacagaccattagttacatggcagaacgggttgttggaacaggatcatttggaattgtattccaggtacctatgtgcttgtccactcactgcaaccatttgaaccgtgagcttcagttaatgcggctaatggaccacccaaacgttgtttccctgaagcattgtttcttctctacgacgagtagagatgagctcttcctcaacctcgttatggagtatgtacccgagactttgtaccgggttttgaagcactatactagttcaaaccagagaatgcctattttctatgtcaaattttacacttaccaaatctttagaggcttggcttatatccatgcagctcctggtgtctgccacagggatttgaaaccacaaaatcttttggttgatcctctcactcatcagtgtaagctgtgcgattttggaagtgcaaaaatattggtgaaaggtgaagcaaacatatcatatatctgctctcgttattaccgagctccagagcttatctttggggccacagagtatacatcctccatagacatatggggccccaaacgaacagcaccatggtctgctggttgtgttttggcagagcttctccttggccagccgttgttcccgggagaaaactctgtggaccagctagtggagatcatcaaggttcttggtactccaactcgagaagagatcagatgcatgaatccaaactacacagacttcagattcccacaaatcaaagctcatccttggcataaggttttccataagcggatgcctccagaaaccattgacctcgcatctcggcttcttcagtattcaccgagcctacgttgcactgcgctggaagcatgtgcacatccatttttcagtgaactacgagagcccaatgcacgtcttccaaacggccgacctctaccaccattgttcaacttcaaacaagagttatctggagcttcactagagcttatagacaggctaatacctgagcacgttaggcggcagatgagtggaggctttccattacaagctggtcat

SEQ ID NO: 19 - protein, 411 aa, Brassica napus
MTSSIPLGHQPPCLAPQPPPQLRDGDALKRRPDMDTDKDMSAAVIEGNDAVTGHIISTTIGGKNGEPKQTISYMAERVVGTGSFGIVFQVPMCLSTHCNHLNRELQLMRLMDHPNVVSLKHCFFSTTSRDELFLNLVMEYVPETLYRVLKHYTSSNQRMPIFYVKFYTYQIFRGLAYIHAAPGVCHRDLKPQNLLVDPLTHQCKLCDFGSAKILVKGEANISYICSRYYRAPELIFGATEYTSSIDIWGPKRTAPWSAGCVLAELLLGQPLFPGENSVDQLVEIIKVLGTPTREEIRCMNPNYTDFRFPQIKAHPWHKVFHKRMPPETIDLASRLLQYSPSLRCTALEACAHPFFSELREPNARLPNGRPLPPLFNFKQELSGASLELIDRLIPEHVRRQMSGGFPLQAGH

SEQ ID NO: 20 - DNA, 1230 bp, Brassica napus
  source 1..1230: mol_type = genomic DNA
atgacatcactatcattgggccctcagcctccggctactgctcagccgccgcagcttcgcgacggagatgcttccaggcgtcgttccgatatggatacagacaaggatatgtctgctgctgtgatagagggaaacgatgctgttacaggccacatcatttctactacaattggaggcaaaaacggtgaacctaaacagaccatcagttacatggccgaacgggttgttggacaaggatcattcggaatcgtgttccaggccaagtgcttggaaactggagaatcagtcgccattaagaaggttttgcaagaccggcgctacaagaatcgtgagctgcagttgatgcgactaatggaccacccaaatgtggtttccttgaagcattgtttcttctctacaacgagtagagatgagctcttcctcaatctcgttatggagtatgtacccgagactttgtaccgggttttgaagcactatactaattcaagccagagaatgcctattttctatgtcaaactctacacataccaaatcttcagaggcttggcttatatccatactgttcctggtgtctgtcacagagatgtgaaaccacaaaatcttttggttgatcctctcactcatcagtgtaagctgtgtgattttggaagtgcaaaagtattggtgaaaggtgaagcaaacatatcatacatttgctctcggtattaccgagctccagagctcatctttggggccacagagtatacatcctccatagacatatggtctgctggttgtgttttggcagagctccttcttggccagccgttgttcccgggagaaaattctgtggaccagctggtagagatcatcaaggttcttggtactccaactcgagaagaaatccgatgcatgaatccaaactacacagacttcagattccctcaaatcaaagctcacccgtggcataaggttttccataagaggatgcctccagaagccattgacctcgcatctcggcttcttcaatactcaccgagcctgcgttacactgcgcttgaagcatgtgcacatccatttttcaatgaactccgtgagccgaatgctcgtcttcctaacggccgacctctaccagccttgttcaacttcaaacaagagttagctggggcttcaccagagctgataaacaggctcataccggagcacataaggcgacagatgagtggaggcttcccatcacagcctggtcat

SEQ ID NO: 21 - protein, 410 aa, Brassica napus
MTSLSLGPQPPATAQPPQLRDGDASRRRSDMDTDKDMSAAVIEGNDAVTGHIISTTIGGKNGEPKQTISYMAERVVGQGSFGIVFQAKCLETGESVAIKKVLQDRRYKNRELQLMRLMDHPNVVSLKHCFFSTTSRDELFLNLVMEYVPETLYRVLKHYTNSSQRMPIFYVKLYTYQIFRGLAYIHTVPGVCHRDVKPQNLLVDPLTHQCKLCDFGSAKVLVKGEANISYICSRYYRAPELIFGATEYTSSIDIWSAGCVLAELLLGQPLFPGENSVDQLVEIIKVLGTPTREEIRCMNPNYTDFRFPQIKAHPWHKVFHKRMPPEAIDLASRLLQYSPSLRYTALEACAHPFFNELREPNARLPNGRPLPALFNFKQELAGASPELINRLIPEHIRRQMSGGFPSQPGH

SEQ ID NO: 22 - DNA, 1140 bp, Brassica napus
  source 1..1140: mol_type = genomic DNA
atggctgacgatagggagatgccggctgctgtagttgatggacatgaccaagtcactggccacataatctccaccaccatcggtggtaaaaacggagaacctaaacagacaataagttacatggcggagcgagttgtcggaacaggctccttcgggatagtgttccaggcgaagtgtctggagactggagaaaccgtggcgataaagaaggtgttgcaagacaggaggtacaagaaccgggagcttcagctgatgcgtgtgatggaccatcctaatgttgtttgtctgaagcattgcttcttctcgaccacgagtaaagacgagctgtttcttaacttggttatggagtatgtccctgagagtttgtaccgagttctgaaacattacagcactgctaaccagaggatgccgcttgtctacgttaaactctatatgtaccagatcttcagaggacttgcttacattcacaatgttgctggagtttgtcacagagatctaaagcctcagaatcttctggttgatcctcttactcatcaagtcaagatctgtgattttggcagtgctaaacagcttgttaaaggtgaagccaacatctcttacatatgctcacggttctaccgtgcacctgaactcatatttggtgccactgagtacacaacttccattgatatctggtctgctggttgtgttctcgctgagcttcttcttggtcagccactattccctggagaaaatgctgtggatcagctcgttgaaataatcaaagttcttggtacaccaactcgaaaagagatccgttgtatgaatccacactacacagacttcaggttcccgcagataaaggcacatccttggcacaagattttccacaaaaggatgcctccagaagcaattgattttgcttcaaggctgcttcagtactctccaagtcttagatgcacagcgcttgaagcttgtgcacatccgttctttgatgagctgagagaaccaaatgctcgtttaccaaacggacggcctttcccacctctcttcaacttcaaacaagaggtagctggagcttcacctgagctggtcaacaagttgattccagaccatatcaagaggcagttgggtctaagcttcttgaatcagtctggaact

SEQ ID NO: 23 - protein, 381 aa, Brassica napus
MADDREMPAAVVDGHDQVTGHIISTTIGGKNGEPKQTISYMAERVVGTGSFGIVFQAKCLETGETVAIKKVLQDRRYKNRELQLMRVMDHPNVVCLKHCFFSTTSKDELFLNLVMEYVPESLYRVLKHYSTANQRMPLVYVKLYMYQIFRGLAYIHNVAGVCHRDLKPQNLLVDPLTHQVKICDFGSAKQLVKGEANISYICSRFYRAPELIFGATEYTTSIDIWSAGCVLAELLLGQPLFPGENAVDQLVEIIKVLGTPTRKEIRCMNPHYTDFRFPQIKAHPWHKIFHKRMPPEAIDFASRLLQYSPSLRCTALEACAHPFFDELREPNARLPNGRPFPPLFNFKQEVAGASPELVNKLIPDHIKRQLGLSFLNQSGTX

SEQ ID NO: 24 - DNA, 1140 bp, Brassica napus
  source 1..1140: mol_type = genomic DNA
atggctgacgataaggagatgccggctgctgtagttgatggacatgaccaagtcactggtcacataatctccaccacaataggaggtaaaaacggagaacctaaacagactataagttacatggcggagcgagtcgtcggcacaggctccttcgggatagtgttccaagcaaagtgtttggagacaggagaaaccgtggcgataaagaaggttttgcaagacaggagatacaagaaccgagagcttcagctgatgcgtgtgatggaccatccgaacgtggttcgtttgaaacattgcttcttctcgaccacgagtaaagacgagcttttccttaatctggttatggagtatgtccctgagagcttgtaccgtgttctgaaacattacagcactgcgaaccagagaatgcctcttgtctacgttaaactctacatgtaccagatctttaggggacttgcttacgttcacaatgttgctggagtttgccatagagatctaaagccgcagaatcttctggttgatcctcttacacatcaagtcaagatatgtgactttggtagtgcgaaacagcttgttaaaggtgaagccaacatatcttacatatgttcaagattctaccgtgcacctgaacttatattcggtgctaccgagtacacaacttcaattgatatctggtctgctggttgtgtccttgctgagcttcttcttggtcagccattattccctggagagaatgctgttgatcagctagttgaaatcatcaaagttcttggtacaccaactcgaaaagagatccgttgtatgaatccacactacacagactttaggttcccacagattaaagcacatccttggcacaagattttccataaacggatgcctccagaagctattgattttgcgtcaaggctgcttcagtactctcctagtcttagatgcacagcgctggaagcttgtgcacatccgttctttgatgaactgagagaaccaaatgctcgtttaccaaacggacggcctttcccgcctctcttcaacttcaaacaggaggtagctggagcatcacctgagctggtcaacaagttgattccagaccatatcaagagacagttgggtctaagtttcttgaatcagtctggaact

SEQ ID NO: 25 - protein, 381 aa, Brassica napus
MADDKEMPAAVVDGHDQVTGHIISTTIGGKNGEPKQTISYMAERVVGTGSFGIVFQAKCLETGETVAIKKVLQDRRYKNRELQLMRVMDHPNVVRLKHCFFSTTSKDELFLNLVMEYVPESLYRVLKHYSTANQRMPLVYVKLYMYQIFRGLAYVHNVAGVCHRDLKPQNLLVDPLTHQVKICDFGSAKQLVKGEANISYICSRFYRAPELIFGATEYTTSIDIWSAGCVLAELLLGQPLFPGENAVDQLVEIIKVLGTPTRKEIRCMNPHYTDFRFPQIKAHPWHKIFHKRMPPEAIDFASRLLQYSPSLRCTALEACAHPFFDELREPNARLPNGRPFPPLFNFKQEVAGASPELVNKLIPDHIKRQLGLSFLNQSGTX

SEQ ID NO: 26 - DNA, 1140 bp, Brassica napus
  source 1..1140: mol_type = genomic DNA
atggctgacgataaggaggtgccgggtgctgtagttaacggacacgatcacgtcactggccacataatctccacaactatcggaggcaaaaacggagaaccaaaacagacgataagttacatggcggagcgtgtcgtcggaacaggctcattcgggatagtcttccaggcgaagtgtttggagaccggagaaaccgtggcgataaagaaggttctgcaagacaggaggtacaagaaccgagagcttcagctgatgcgtgttatggaccatcctaatgtggtttgtttgaagcattgcttcttctccaccactagtaaagacgagctgtttctcaacttggttatggagtatgtacccgagagcttgtaccgtgttctgaaacattacagcactgctaaccagagaatgcctcttgtctatgttaaactctacatgtaccagatcttcaggggacttgcttatatgcacaatgttgctgaagtttgtcacagagatctaaagcctcaaaatcttctggttgatcctcttactcatcaagtcaagatctgtgactttggcagtgctaaacagcttgttaaaggtgaagccaacatctcttacatatgttcaagattctaccgtgcaccagagctcatatttggtgccactgagtacacaacttccattgatatctggtctgctggttgtgttcttgctgagcttctccttggtcagccattattccctggagaaaatgctgtggatcagctcgttgaaatcatcaaagttcttggtacaccaactcgaaaagagatccgttgcatgaatccacattacacggactttaggttcccacagataaaggcacacccttggcacaagattttccataaaaggatgcctccagaagcgattgatttcgcatcgaggctgcttcagtactctccaagtcttagatgcacagctcttgaagcttgtgcacatccgttctttgatgaactgagagaaccaaatgctcgtttaccaaacggacggcctttcccgccaatcttcaacttcaaacaagaggtagctggagcatcacctgagctggtcaacaagttgattccggaccatatcaagagacagttgggtctaagtttcttgaatcagtctggaact

SEQ ID NO: 27 - protein, 381 aa, Brassica napus
MADDKEVPGAVVNGHDHVTGHIISTTIGGKNGEPKQTISYMAERVVGTGSFGIVFQAKCLETGETVAIKKVLQDRRYKNRELQLMRVMDHPNVVCLKHCFFSTTSKDELFLNLVMEYVPESLYRVLKHYSTANQRMPLVYVKLYMYQIFRGLAYMHNVAEVCHRDLKPQNLLVDPLTHQVKICDFGSAKQLVKGEANISYICSRFYRAPELIFGATEYTTSIDIWSAGCVLAELLLGQPLFPGENAVDQLVEIIKVLGTPTRKEIRCMNPHYTDFRFPQIKAHPWHKIFHKRMPPEAIDFASRLLQYSPSLRCTALEACAHPFFDELREPNARLPNGRPFPPIFNFKQEVAGASPELVNKLIPDHIKRQLGLSFLNQSGTX

SEQ ID NO: 28 - DNA, 1140 bp, Brassica napus
  source 1..1140: mol_type = genomic DNA
atggctgacgataaggaggtgcctgctgctgtagttaacggacacgatcaagtcactggccacataatctccacaactatcggaggcaaaaacggagaaccaaaacagacgataagttacatggcggagcgagtcgtcggaacaggctccttcgggatagtcttccaggccaagtgtttggagaccggagaaaccgtggcgataaagaaggttctgcaagacaggaggtacaagaaccgagagcttcagctgatgcgcgtcatggaccatcctaatgtggtttgtttgaagcattgcttcttctccaccactagtaaagacgagctgtttctcaacttggttatggagtatgtacccgagagcttgtaccgtgttctgaaacattacagcactgccaaccagagaatgcctcttgtctatgttaaactctacatgtaccagatcttcaggggacttgcttatatgcacaatgttgctggagtttgtcacagagatctaaagcctcaaaatcttctggttgatcctctgactcatcaagtcaagatctgtgactttgggagtgctaaacagcttgttaaaggtgaagccaacatctcttacatatgttcaagattctaccgtgcacccgagctcatattcggtgccaccgagtacacaacttccattgatatctggtctgctggttgtgttcttgctgagcttcttctcggtcagccattattccctggagaaaatgctgtggatcagcttgttgaaatcatcaaagttcttggtacaccaactcgaaaagagatccgttgtatgaatccacattacacagactttaggttccctcagataaaggcacacccttggcacaagattttccataaaaggatgcctccagaagctattgatttcgcatcaaggctgcttcagtactctccaagtcttagatgcacagcgctggaagcatgtgcacatccgttctttgatgagctcagagaaccaaatgctcgtttaccaaacggacggcctttcccgcctatcttcaacttcaaacaagaggtagctggagcatcacctgagctggtcaacaagttgattccagaccatatcaagagacagttgggtctgagtttcttgaatcagtctggaact

SEQ ID NO: 29 - protein, 381 aa, Brassica napus
MADDKEVPAAVVNGHDQVTGHIISTTIGGKNGEPKQTISYMAERVVGTGSFGIVFQAKCLETGETVAIKKVLQDRRYKNRELQLMRVMDHPNVVCLKHCFFSTTSKDELFLNLVMEYVPESLYRVLKHYSTANQRMPLVYVKLYMYQIFRGLAYMHNVAGVCHRDLKPQNLLVDPLTHQVKICDFGSAKQLVKGEANISYICSRFYRAPELIFGATEYTTSIDIWSAGCVLAELLLGQPLFPGENAVDQLVEIIKVLGTPTRKEIRCMNPHYTDFRFPQIKAHPWHKIFHKRMPPEAIDFASRLLQYSPSLRCTALEACAHPFFDELREPNARLPNGRPFPPIFNFKQEVAGASPELVNKLIPDHIKRQLGLSFLNQSGTX

SEQ ID NO: 30 - DNA, 1233 bp, Brassica napus
  source 1..1233: mol_type = genomic DNA
atgacatcctccataccattgggtcatcagcctccgtgtctagctccgcagccgccgccgcagctgcgcgacggagatgctttgaaacgtcgtcctgatatggatacagacaaggatatgtctgctgctgttatagagggcaatgatgctgttaccggtcacatcatttctactaccatcggaggcaaaaacggcgaacctaaacagaccattagttacatggcagaacgggttgttggaacaggatcatttggaattgtattccaggtacctatgtgcttgtccactcactgcaaccatttgaaccgtgagcttcagttaatgcggctaatggaccacccaaacgttgtttccctgaagcattgtttcttctctacgacgagtagagatgagctcttcctcaacctcgttatggagtatgtacccgagactttgtaccgggttttgaagcactatactagttcaaaccagagaatgcctattttctatgtcaaattttacacttaccaaatctttagaggcttggcttatatccatgcagctcctggtgtctgccacagggatttgaaaccacaaaatcttttggttgatcctctcactcatcagtgtaagctgtgcgattttggaagtgcaaaaatattggtgaaaggtgaagcaaacatatcatatatctgctctcgttattaccgagctccagagcttatctttggggccacagagtatacatcctccatagacatatggggccccaaacgaacagcaccatggtctgctggttgtgttttggcagagcttctccttggccagccgttgttcccgggagaaaactctgtggaccagctagtggagatcatcaaggttcttggtactccaactcgaaaagagatcagatgcatgaatccaaactacacagacttcagattcccacaaatcaaagctcatccttggcataaggttttccataagcggatgcctccagaaaccattgacctcgcatctcggcttcttcagtattcaccgagcctacgttgcactgcgctggaagcatgtgcacatccatttttcagtgaactacgagagcccaatgcacgtcttccaaacggccgacctctaccaccattgttcaacttcaaacaagagttatctggagcttcactagagcttatagacaggctaatacctgagcacgttaggcggcagatgagtggaggctttccattacaagctggtcat

SEQ ID NO: 31 - protein, 412 aa, Brassica napus
MTSSIPLGHQPPCLAPQPPPQLRDGDALKRRPDMDTDKDMSAAVIEGNDAVTGHIISTTIGGKNGEPKQTISYMAERVVGTGSFGIVFQVPMCLSTHCNHLNRELQLMRLMDHPNVVSLKHCFFSTTSRDELFLNLVMEYVPETLYRVLKHYTSSNQRMPIFYVKFYTYQIFRGLAYIHAAPGVCHRDLKPQNLLVDPLTHQCKLCDFGSAKILVKGEANISYICSRYYRAPELIFGATEYTSSIDIWGPKRTAPWSAGCVLAELLLGQPLFPGENSVDQLVEIIKVLGTPTRKEIRCMNPNYTDFRFPQIKAHPWHKVFHKRMPPETIDLASRLLQYSPSLRCTALEACAHPFFSELREPNARLPNGRPLPPLFNFKQELSGASLELIDRLIPEHVRRQMSGGFPLQAGHX

SEQ ID NO: 32 - DNA, 1230 bp, Brassica napus
  source 1..1230: mol_type = genomic DNA
atgacatcactatcattgggccctcagcctccggctactgctcagccgccgcagcttcgcgacggagatgcttccaggcgtcgttccgatatggatacagacaaggatatgtctgctgctgtgatagagggaaacgatgctgttacaggccacatcatttctactacaattggaggcaaaaacggtgaacctaaacagaccatcagttacatggccgaacgggttgttggacaaggatcattcggaatcgtgttccaggccaagtgcttggaaactggagaatcagtcgccattaagaaggttttgcaagaccggcgctacaagaatcgtgagctgcagttgatgcgactaatggaccacccaaatgtggtttccttgaagcattgtttcttctctacaacgagtagagatgagctcttcctcaatctcgttatggagtatgtacccgagactttgtaccgggttttgaagcactatactaattcaagccagagaatgcctattttctatgtcaaactctacacataccaaatcttcagaggcttggcttatatccatactgttcctggtgtctgtcacagagatgtgaaaccacaaaatcttttggttgatcctctcactcatcagtgtaagctgtgtgattttggaagtgcaaaagtattggtgaaaggtgaagcaaacatatcatacatttgctctcggtattaccgagctccagagctcatctttggggccacagagtatacatcctccatagacatatggtctgctggttgtgttttggcagagctccttcttggccagccgttgttcccgggagaaaattctgtggaccagctggtagagatcatcaaggttcttggtactccaactcgaaaagaaatccgatgcatgaatccaaactacacagacttcagattccctcaaatcaaagctcacccgtggcataaggttttccataagaggatgcctccagaagccattgacctcgcatctcggcttcttcaatactcaccgagcctgcgttacactgcgcttgaagcatgtgcacatccatttttcaatgaactccgtgagccgaatgctcgtcttcctaacggccgacctctaccagccttgttcaacttcaaacaagagttagctggggcttcaccagagctgataaacaggctcataccggagcacataaggcgacagatgagtggaggcttcccatcacagcctggtcat

SEQ ID NO: 33 - protein, 411 aa, Brassica napus
MTSLSLGPQPPATAQPPQLRDGDASRRRSDMDTDKDMSAAVIEGNDAVTGHIISTTIGGKNGEPKQTISYMAERVVGQGSFGIVFQAKCLETGESVAIKKVLQDRRYKNRELQLMRLMDHPNVVSLKHCFFSTTSRDELFLNLVMEYVPETLYRVLKHYTNSSQRMPIFYVKLYTYQIFRGLAYIHTVPGVCHRDVKPQNLLVDPLTHQCKLCDFGSAKVLVKGEANISYICSRYYRAPELIFGATEYTSSIDIWSAGCVLAELLLGQPLFPGENSVDQLVEIIKVLGTPTRKEIRCMNPNYTDFRFPQIKAHPWHKVFHKRMPPEAIDLASRLLQYSPSLRYTALEACAHPFFNELREPNARLPNGRPLPALFNFKQELAGASPELINRLIPEHIRRQMSGGFPSQPGHX

SEQ ID NO: 34 - DNA, 1140 bp, Brassica napus
  source 1..1140: mol_type = genomic DNA
atggctgccgataaggagatgccagctgctgtagttgctgggcatgatcaagtcactggtcacataatctccaccacaataggaggaaaaaacggagaacctaaacagacaataagttacatggcggagcgagtcgtcggcacaggttccttcgggatagtgttccaagcaaagtgtttggagacaggagaaaccgtagcgataaagaaagttctgcaagacaggagatacaagaaccgagagcttcagctgatgcgcgtgatggaccatccgaacgtggttcgtttgaagcattgcttcttctcgaccacgagtaaagacgagcttttccttaacttggttatggagtatgtccccgagagcttgtaccgtgttctcaaacattacagcaccgcgaaccagagaatgcctcttgtctacgttaaactctacatgtaccagatctttaggggacttgcttacgttcacaatgttgctggtgtttgccatagagatctaaagcctcaaaatcttctggttgatcctctaactcatcaagtcaagatctgtgactttggcagtgcgaaacagcttgttaaaggtgaagccaacatttcttacatatgttcaagattctaccgagcacctgaactcatatttggtgccactgagtacacaacatcaattgatatctggtctgctggttgtgtcctcgctgagcttcttcttggtcagccattattccctggagagaatgctgttgatcagctagttgaaatcatcaaagttcttggtacaccaactcgaaaagagatccgttgtatgaatccacactacacagactttaggttcccgcagataaaagcacatccttggcacaagattttccacaaaagaatgcctccagaagctcttgattttgcgtcaaggctgcttcagtactctcctagtcttagatgcacagcgctggaagcttgtgcacatcctttctttgatgaactgagagaaccaaatgcttgtttaccaaacggacggcctttcccgcctctcttcaacttcaaacaggaggttgctggagcatcacctgagctggtgaacaagttgattccagaccatatcaagagacaattgggtctaagtttcttgaatcagtctggaact

SEQ ID NO: 35 - protein, 381 aa, Brassica napus
MAADKEMPAAVVAGHDQVTGHIISTTIGGKNGEPKQTISYMAERVVGTGSFGIVFQAKCLETGETVAIKKVLQDRRYKNRELQLMRVMDHPNVVRLKHCFFSTTSKDELFLNLVMEYVPESLYRVLKHYSTANQRMPLVYVKLYMYQIFRGLAYVHNVAGVCHRDLKPQNLLVDPLTHQVKICDFGSAKQLVKGEANISYICSRFYRAPELIFGATEYTTSIDIWSAGCVLAELLLGQPLFPGENAVDQLVEIIKVLGTPTRKEIRCMNPHYTDFRFPQIKAHPWHKIFHKRMPPEALDFASRLLQYSPSLRCTALEACAHPFFDELREPNACLPNGRPFPPLFNFKQEVAGASPELVNKLIPDHIKRQLGLSFLNQSGTX

SEQ ID NO: 36 - DNA, 186 bp, synthetic construct
  source 1..186: mol_type = other DNA
catgcatcggatttcttctcgttttagagctagaaatagcaagttaaaataaggctagtccgttatcaacttgaaaaagtggcaccgagtcggtgcccaacccgaaaagaaatccgatgccggcatggtcccagcctcctcgctggcgccggctgggcaacatgcttcggcatggcgaatgggact